European Patent Application EP 4 644 417 A1, published November 5, 2025. Title: Affibody specifically binding to CD137 and Use thereof. Applicant: AbClon Inc. The sequence listing filed with the application follows.

SEQUENCE LISTING (39 sequences)

SEQ ID NO: 1 - protein, 58 aa, synthetic construct
VDNKFNKEVCRAMEEIGMLPNLNAHQLAAFIWSLPDDPSQSANLLAEAKKLNDAQAPK

SEQ ID NO: 2 - protein, 58 aa, synthetic construct
VDNKFNKEECTAYFEIANLPNLNTAQLAAFIWSLRDDPSQSANLLAEAKKLNDAQAPK

SEQ ID NO: 3 - protein, 58 aa, synthetic construct
VDNKFNKEVCTAFDEIAHLPNLNVHQLAAFIWSLTDDPSQSANLLAEAKKLNDAQAPK

SEQ ID NO: 4 - protein, 58 aa, synthetic construct
VDNKFNKEYCFAMDEIASLPNLNPHQLAAFIWSLDDDPSQSANLLAEAKKLNDAQAPK

SEQ ID NO: 5 - protein, 58 aa, synthetic construct
VDNKFNKEECSAMQEISMLPNLNPHQFAAFIWSLMDDPSQSANLLAEAKKLNDAQAPK

SEQ ID NO: 6 - protein, 58 aa, synthetic construct
VDNKFNKEQCWAIAEIAGLPNLNVHQLAAFIWSLSDDPSQSANLLAEAKKLNDAQAPK

SEQ ID NO: 7 - protein, 58 aa, synthetic construct
VDNKFNKEFCMASTEIGGLPNLNVHQLAAFIWSLSDDPSQSANLLAEAKKLNDAQAPK

SEQ ID NO: 8 - protein, 58 aa, synthetic construct
VDNKFNKEFCFAIGEIATLPNLNAHQIAAFIWSLDDDPSQSANLLAEAKKLNDAQAPK

SEQ ID NO: 9 - DNA, 174 bp, synthetic construct
  source 1..174: mol_type = other DNA
gtggacaacaagttcaacaaggaggtttgccgtgccatggaagagattggtatgctgcccaacctgaacgctcatcagctggctgccttcatttggtccctgccggacgacccttcccagtccgccaacctgctggccgaggccaagaagctgaacgacgcccaggctcccaag

SEQ ID NO: 10 - DNA, 174 bp, synthetic construct
  source 1..174: mol_type = other DNA
gtggacaacaagttcaacaaggaggaatgcactgcctacttcgagattgctaacctgcccaacctgaacactgctcagctggctgccttcatttggtccctgcgtgacgacccttcccagtccgccaacctgctggccgaggccaagaagctgaacgacgcccaggctcccaag

SEQ ID NO: 11 - DNA, 174 bp, synthetic construct
  source 1..174: mol_type = other DNA
gtggacaacaagttcaacaaggaggtttgcactgccttcgacgagattgctcatctgcccaacctgaacgttcatcagctggctgccttcatttggtccctgactgacgacccttcccagtccgccaacctgctggccgaggccaagaagctgaacgacgcccaggctcccaag

SEQ ID NO: 12 - DNA, 174 bp, synthetic construct
  source 1..174: mol_type = other DNA
gtggacaacaagttcaacaaggagtactgcttcgccatggacgagattgcttctctgcccaacctgaacccgcatcagctggctgccttcatttggtccctggacgacgacccttcccagtccgccaacctgctggccgaggccaagaagctgaacgacgcccaggctcccaag

SEQ ID NO: 13 - DNA, 174 bp, synthetic construct
  source 1..174: mol_type = other DNA
gtggacaacaagttcaacaaggaggaatgctctgccatgcaggagatttctatgctgcccaacctgaacccgcatcagttcgctgccttcatttggtccctgatggacgacccttcccagtccgccaacctgctggccgaggccaagaagctgaacgacgcccaggctcccaag

SEQ ID NO: 14 - DNA, 174 bp, synthetic construct
  source 1..174: mol_type = other DNA
gtggacaacaagttcaacaaggagcagtgctgggccatcgctgagattgctggtctgcccaacctgaacgttcatcagctggctgccttcatttggtccctgtctgacgacccttcccagtccgccaacctgctggccgaggccaagaagctgaacgacgcccaggctcccaag

SEQ ID NO: 15 - DNA, 174 bp, synthetic construct
  source 1..174: mol_type = other DNA
gtggacaacaagttcaacaaggagttctgcatggcctctactgagattggtggtctgcccaacctgaacgttcatcagctggctgccttcatttggtccctgtctgacgacccttcccagtccgccaacctgctggccgaggccaagaagctgaacgacgcccaggctcccaag

SEQ ID NO: 16 - DNA, 174 bp, synthetic construct
  source 1..174: mol_type = other DNA
gtggacaacaagttcaacaaggagttctgcttcgccatcggtgagattgctactctgcccaacctgaacgctcaccagatcgctgccttcatttggtccctggacgacgacccttcccagtccgccaacctgctggccgaggccaagaagctgaacgacgcccaggctcccaag

SEQ ID NO: 17 - protein, 6 aa, synthetic construct
TRYWLH

SEQ ID NO: 18 - protein, 17 aa, synthetic construct
EINPSSGRTNYNEKFKS

SEQ ID NO: 19 - protein, 11 aa, synthetic construct
WDYDEGTWFAY

SEQ ID NO: 20 - protein, 11 aa, synthetic construct
RASENIYSYLA

SEQ ID NO: 21 - protein, 7 aa, synthetic construct
NARTLVE

SEQ ID NO: 22 - protein, 9 aa, synthetic construct
QHHYGPPYT

SEQ ID NO: 23 - protein, 120 aa, synthetic construct
QVQLVQSGAEVKKPGASVKVSCKASGYTFTRYWLHWVRQAPGQGLEWIGEINPSSGRTNYNEKFKSRATLTVDKSISTAYMELSRLRSDDTAVYYCARWDYDEGTWFAYWGQGTLVTVSS

SEQ ID NO: 24 - protein, 107 aa, synthetic construct
DIQMTQSPSFLSASVGDRVTITCRASENIYSYLAWYQQKPGKAPKLLVYNARTLVEGVPSRFSGSGSGTEFTLTISSLQPEDFATYYCQHHYGPPYTFGQGTKVEIK

SEQ ID NO: 25 - DNA, 360 bp, synthetic construct
  source 1..360: mol_type = other DNA
caggttcagctcgtgcaatcaggcgctgaggttaaaaagccaggagccagtgtcaaagtgtcttgtaaggcctccgggtataccttcacaaggtactggctgcactgggtgagacaagcacccggtcagggccttgagtggatcggggaaattaatcctagcagtggcagaaccaattataacgagaagttcaagtctcgcgccactctgactgtagataaaagcatcagcacggcctacatggagctgtctagactgagatccgacgataccgctgtctactactgcgcgagatgggactatgacgaaggtacatggtttgcatattggggccagggaaccttggtgacagtgtcatcc

SEQ ID NO: 26 - DNA, 321 bp, synthetic construct
  source 1..321: mol_type = other DNA
gacatccagatgacccagtcacctagcttcctgtctgcttctgtcggggacagagtgactatcacttgtcgcgcctccgagaacatatactcctatctcgcttggtaccaacagaagcccgggaaggccccaaaacttctggtatacaatgcccggaccctggttgagggcgtgccttcaaggttcagtgggagcggctccggaaccgaattcacgttgacaattagtagcctgcaaccggaggattttgcaacatactattgccagcaccattacggccccccatatacctttggacagggtacaaaggtggaaattaaa

SEQ ID NO: 27 - protein, 163 aa, synthetic construct
LQDPCSNCPAGTFCDNNRNQICSPCPPNSFSSAGGQRTCDICRQCKGVFRTRKECSSTSNAECDCTPGFHCLGAGCSMCEQDCKQGQELTKKGCKDCCFGTFNDQKRGICRPWTNCSLDGKSVLVNGTKERDVVCGPSPADLSPGASSVTPPAPAREPGHSPQ

SEQ ID NO: 28 - protein, 447 aa, synthetic construct
EVQLVESGGGLVQPGGSLRLSCAASGFNIKDTYIHWVRQAPGKGLEWVARIYPTNGYTRYADSVKGRFTISADTSKNTAYLQMNSLRAEDTAVYYCSRWGGDGFYAMDYWGQGTLVTVSSASTKGPSVFPLAPCSRSTSESTAALGCLVKDYFPEPVTVSWNSGALTSGVHTFPAVLQSSGLYSLSSVVTVPSSSLGTKTYTCNVDHKPSNTKVDKRVESKYGPPCPPCPAPEFLGGPSVFLFPPKPKDTLMISRTPEVTCVVVDVSQEDPEVQFNWYVDGVEVHNAKTKPREEQFNSTYRVVSVLTVLHQDWLNGKEYKCKVSNKGLPSSIEKTISKAKGQPREPQVYTLPPSQEEMTKNQVSLTCLVKGFYPSDIAVEWESNGQPENNYKTTPPVLDSDGSFFLYSRLTVDKSRWQEGNVFSCSVMHEALHNHYTQKSLSLSLGK

SEQ ID NO: 29 - protein, 214 aa, synthetic construct
DIQMTQSPSSLSASVGDRVTITCRASQDVNTAVAWYQQKPGKAPKLLIYSASFLYSGVPSRFSGSRSGTDFTLTISSLQPEDFATYYCQQHYTTPPTFGQGTKVEIKRTVAAPSVFIFPPSDEQLKSGTASVVCLLNNFYPREAKVQWKVDNALQSGNSQESVTEQDSKDSTYSLSSTLTLSKADYEKHKVYACEVTHQGLSSPVTKSFNRGEC

SEQ ID NO: 30 - protein, 5 aa, synthetic construct
SYTMS

SEQ ID NO: 31 - protein, 16 aa, synthetic construct
YISAGGGSTYYPDTVK

SEQ ID NO: 32 - protein, 10 aa, synthetic construct
HLGGTASFDY

SEQ ID NO: 33 - protein, 11 aa, synthetic construct
LASQTIGTWLA

SEQ ID NO: 34 - protein, 6 aa, synthetic construct
ATSLAD

SEQ ID NO: 35 - protein, 9 aa, synthetic construct
QQNAYAPWT

SEQ ID NO: 36 - protein, 446 aa, synthetic construct
EVQLVESGGGLVQPGGSLRLSCAASGFTFSSYTMSWVRQAPGKGLEWVAYISAGGGSTYYPDTVKGRFTISRDNAKNSLYLQMNSLRAEDTAVYYCARHLGGTASFDYWGQGTLVTVSSASTKGPSVFPLAPCSRSTSESTAALGCLVKDYFPEPVTVSWNSGALTSGVHTFPAVLQSSGLYSLSSVVTVPSSSLGTKTYTCNVDHKPSNTKVDKRVESKYGPPCPPCPAPEFLGGPSVFLFPPKPKDTLMISRTPEVTCVVVDVSQEDPEVQFNWYVDGVEVHNAKTKPREEQFNSTYRVVSVLTVLHQDWLNGKEYKCKVSNKGLPSSIEKTISKAKGQPREPQVYTLPPSQEEMTKNQVSLTCLVKGFYPSDIAVEWESNGQPENNYKTTPPVLDSDGSFFLYSRLTVDKSRWQEGNVFSCSVMHEALHNHYTQKSLSLSLGK

SEQ ID NO: 37 - protein, 214 aa, synthetic construct
DIQMTQSPSSLSASVGDRVTITCLASQTIGTWLAWYQQKPGKAPKLLIYVATSLADGVPSRFSGSGSGTDFTLTISSLQPEDFATYYCQQNAYAPWTFGQGTKVEIKRTVAAPSVFIFPPSDEQLKSGTASVVCLLNNFYPREAKVQWKVDNALQSGNSQESVTEQDSKDSTYSLSSTLTLSKADYEKHKVYACEVTHQGLSSPVTKSFNRGEC

SEQ ID NO: 38 - protein, 447 aa, synthetic construct
EVKLQESGPGLVAPSQSLSVTCTVSGVSLPDYGVSWIRQPPRKGLEWLGVIWGSETTYYNSALKSRLTIIKDNSKSQVFLKMNSLQTDDTAIYYCAKHYYYGGSYAMDYWGQGTSVTVSSASTKGPSVFPLAPCSRSTSESTAALGCLVKDYFPEPVTVSWNSGALTSGVHTFPAVLQSSGLYSLSSVVTVPSSSLGTKTYTCNVDHKPSNTKVDKRVESKYGPPCPPCPAPEFLGGPSVFLFPPKPKDTLMISRTPEVTCVVVDVSQEDPEVQFNWYVDGVEVHNAKTKPREEQFNSTYRVVSVLTVLHQDWLNGKEYKCKVSNKGLPSSIEKTISKAKGQPREPQVYTLPPSQEEMTKNQVSLTCLVKGFYPSDIAVEWESNGQPENNYKTTPPVLDSDGSFFLYSRLTVDKSRWQEGNVFSCSVMHEALHNHYTQKSLSLSLGK

SEQ ID NO: 39 - protein, 214 aa, synthetic construct
DIQMTQTTSSLSASLGDRVTISCRASQDISKYLNWYQQKPDGTVKLLIYHTSRLHSGVPSRFSGSGSGTDYSLTISNLEQEDIATYFCQQGNTLPYTFGGGTKLEITRTVAAPSVFIFPPSDEQLKSGTASVVCLLNNFYPREAKVQWKVDNALQSGNSQESVTEQDSKDSTYSLSSTLTLSKADYEKHKVYACEVTHQGLSSPVTKSFNRGEC